European Patent Specification EP 4 028 543 B1, published June 12, 2024. Title: "Method for preparing an RNA sample for sequencing and kit thereof". Applicant: Immagina Biotechnology S.r.l. The sequence listing filed with the application follows.

SEQUENCE LISTING (5 sequences)

SEQ ID NO: 1 - RNA, 30 nt, artificial
  GFP fragment
  misc_feature (1)..(1): phosphate group
  misc_feature (30)..(30): phosphate group
auucuuguugaauuagauggcgauguuaau

SEQ ID NO: 2 - DNA, 958 bp, artificial
  GFP fragment
gtaagtatcaaggttacaagacaggtttaaggaggccaatagaaactgggcttgtcgagacagagaagattcttgcgtttctgataggcacctattggtcttactgacatccactttgcctttctctccacaggggtaccgaagccgctagcgctaccggtcgccaccatgcccgccatgaagatcgagtgccgcatcaccggcaccctgaacggcgtggagttcgagctggtgggcggcggagagggcacccccgagcagggccgcatgaccaacaagatgaagagcaccaaaggcgccctgaccttcagcccctacctgctgagccacgtgatgggctacggcttctaccacttcggcacctaccccagcggctacgagaaccccttcctgcacgccatcaacaacggcggctacaccaacacccgcatcgagaagtacgaggacggcggcgtgctgcacgtgagcttcagctaccgctacgaggccggccgcgtgatcggcgacttcaaggtggtgggcaccggcttccccgaggacagcgtgatcttcaccgacaagatcatccgcagcaacgccaccgtggagcacctgcaccccatgggcgataacgtgctggtgggcagcttcgcccgcaccttcagcctgcgcgacggcggctactacagcttcgtggtggacagccacatgcacttcaagagcgccatccaccccagcatcctgcagaacgggggccccatgttcgccttccgccgcgtggaggagctgcacagcaacaccgagctgggcatcgtggagtaccagcacgccttcaagacccccatcgccttcgccagatctcgagctcgatgagtttggacaaaccacaactagaatgcagtgaaaaaaatgctttatttgtgaaatttgtgatgctattgctttatttgtaaccattataagctgcaataaacaagtt

SEQ ID NO: 3 - RNA, 109 nt, artificial
  Linker R
cuggucacuucuucaagaccgcugguauccaaauuguugcugaugacuugacugucaccaacccagcuagaauugcuaccgccaucgaaaagaaggcugcugacgcuuu

SEQ ID NO: 4 - DNA, 18 bp, artificial
  RT-RCA Fw (primer second strand cDNA synthesis)
tggtcacttcttcaagac

SEQ ID NO: 5 - DNA, 18 bp, artificial
  RT-RCA Rev (primer second strand cDNA synthesis)
gtcagcagccttcttttc